European Patent Application EP 4 501 918 A1, published February 5, 2025. Title: 3-phenylisoxazole derivatives and pharmaceutical compositions for preventing or treating eye disease containing the same as an active ingredient. Applicant: VASTHERA Co., Ltd. The sequence listing filed with the application follows.

SEQUENCE LISTING (8 sequences)

SEQ ID NO: 1 - DNA, 20 bp, synthetic construct
  source 1..20: mol_type = other DNA
gaggatgaggtggaacgtgt

SEQ ID NO: 2 - DNA, 20 bp, synthetic construct
  source 1..20: mol_type = other DNA
tcttcagtcgctccaggtct

SEQ ID NO: 3 - DNA, 20 bp, synthetic construct
  source 1..20: mol_type = other DNA
ccacctccagggacaggata

SEQ ID NO: 4 - DNA, 20 bp, synthetic construct
  source 1..20: mol_type = other DNA
aacacgcaggacaggtacag

SEQ ID NO: 5 - DNA, 20 bp, synthetic construct
  source 1..20: mol_type = other DNA
ccccaggagaagattccaaa

SEQ ID NO: 6 - DNA, 20 bp, synthetic construct
  source 1..20: mol_type = other DNA
ttgttttctgccagtgcctc

SEQ ID NO: 7 - DNA, 26 bp, synthetic construct
  source 1..26: mol_type = other DNA
tgaattacggaataatgagttagaac

SEQ ID NO: 8 - DNA, 23 bp, synthetic construct
  source 1..23: mol_type = other DNA
tcaaccagcaagaaattactaat